European Patent Application EP 4 155 320 A1, published March 29, 2023. Title: ANTI-B7H4 ANTIBODY, BISPECIFIC ANTIBODY AND USE THEREOF. Applicant: Nona Biosciences (Suzhou) Co,. Ltd. Application 21834047.9. The sequence listing filed with the application follows.

SEQUENCE LISTING (135 sequences)

SEQ ID NO: 1 - protein, 25 aa, Artificial Sequence
  Synthetic
EVQLVQSGAEVKKPGASVKVSCKAS

SEQ ID NO: 2 - protein, 25 aa, Artificial Sequence
  Synthetic
EVQLVESGGGLVQPGGSLKLSCAAS

SEQ ID NO: 3 - protein, 25 aa, Artificial Sequence
  Synthetic
QVQLVESGGGVVQPGRSLRLSCAAS

SEQ ID NO: 4 - protein, 25 aa, Artificial Sequence
  Synthetic
EVQLLESGGGLVQPGGSLRLSCAAS

SEQ ID NO: 5 - protein, 25 aa, Artificial Sequence
  Synthetic
QVQLVQSGAEVKKPGSSMRVSCKAS

SEQ ID NO: 6 - protein, 25 aa, Artificial Sequence
  Synthetic
QLQLQESGPGLVKPSETLSLTCTVS

SEQ ID NO: 7 - protein, 7 aa, Artificial Sequence
  Synthetic
GYTFTSY

SEQ ID NO: 8 - protein, 7 aa, Artificial Sequence
  Synthetic
GFTFNTY

SEQ ID NO: 9 - protein, 7 aa, Artificial Sequence
  Synthetic
GFTFRSF

SEQ ID NO: 10 - protein, 7 aa, Artificial Sequence
  Synthetic
GFTFSTY

SEQ ID NO: 11 - protein, 7 aa, Artificial Sequence
  Synthetic
EDTFSSY

SEQ ID NO: 12 - protein, 9 aa, Artificial Sequence
  Synthetic
GGSIKSGSY

SEQ ID NO: 13 - protein, 19 aa, Artificial Sequence
  Synthetic
WIGWVRQAPGQGLEWIGDI

SEQ ID NO: 14 - protein, 19 aa, Artificial Sequence
  Synthetic
AMNWVRQASGKGLEWVGRI

SEQ ID NO: 15 - protein, 19 aa, Artificial Sequence
  Synthetic
GMHWVRQAPGKGLEWVAVI

SEQ ID NO: 16 - protein, 19 aa, Artificial Sequence
  Synthetic
AMNWVRQAPGKGLEWVSRI

SEQ ID NO: 17 - protein, 19 aa, Artificial Sequence
  Synthetic
AISWVRQAPGQGLEWMGGT

SEQ ID NO: 18 - protein, 19 aa, Artificial Sequence
  Synthetic
YWGWIRQPPGKGLEWIGNI

SEQ ID NO: 19 - protein, 6 aa, Artificial Sequence
  Synthetic
YPGGGY

SEQ ID NO: 20 - protein, 8 aa, Artificial Sequence
  Synthetic
RSKYNNYA

SEQ ID NO: 21 - protein, 6 aa, Artificial Sequence
  Synthetic
SYDGSN

SEQ ID NO: 22 - protein, 6 aa, Artificial Sequence
  Synthetic
APIFGT

SEQ ID NO: 23 - protein, 6 aa, Artificial Sequence
  Synthetic
SYEGSN

SEQ ID NO: 24 - protein, 6 aa, Artificial Sequence
  Synthetic
SYDASN

SEQ ID NO: 25 - protein, 5 aa, Artificial Sequence
  Synthetic
YYSGS

SEQ ID NO: 26 - protein, 41 aa, Artificial Sequence
  Synthetic
TNYNEKFKGRVTITRDTSTSTAYLELSSLRSEDTAVYYCAR

SEQ ID NO: 27 - protein, 41 aa, Artificial Sequence
  Synthetic
TYYADSVKDRFTISRDDSKSTLYLQMNSLKTEDTAVYYCVR

SEQ ID NO: 28 - protein, 41 aa, Artificial Sequence
  Synthetic
EYYADSVKGRFIISRDNSKDTLYLQMNSLRAGDTAVYYCAK

SEQ ID NO: 29 - protein, 41 aa, Artificial Sequence
  Synthetic
TYYADSVKDRFTISRDDSKSTLYLQMNSLRAEDTAVYYCVR

SEQ ID NO: 30 - protein, 41 aa, Artificial Sequence
  Synthetic
TNYAQKFQGRVTITADKSTSTAYMELSSLRSEDTAVYYCAR

SEQ ID NO: 31 - protein, 41 aa, Artificial Sequence
  Synthetic
TYYNPSLRSRVTISVDTSKNQFSLKLSSVTAADTAVYYCAR

SEQ ID NO: 32 - protein, 41 aa, Artificial Sequence
  Synthetic
TYYADSVKDRFTISRDDSKNTAYLQMNSLKTEDTAVYYCTR

SEQ ID NO: 33 - protein, 12 aa, Artificial Sequence
  Synthetic
LAGSSYRGAMDS

SEQ ID NO: 34 - protein, 14 aa, Artificial Sequence
  Synthetic
HGNFGNSYVSWFAY

SEQ ID NO: 35 - protein, 10 aa, Artificial Sequence
  Synthetic
GGGLRWYFAY

SEQ ID NO: 36 - protein, 7 aa, Artificial Sequence
  Synthetic
GGPYFDY

SEQ ID NO: 37 - protein, 10 aa, Artificial Sequence
  Synthetic
EGSYPNQFDP

SEQ ID NO: 38 - protein, 10 aa, Artificial Sequence
  Synthetic
GGALRWYFAY

SEQ ID NO: 39 - protein, 11 aa, Artificial Sequence
  Synthetic
WGQGTLVTVSS

SEQ ID NO: 40 - protein, 23 aa, Artificial Sequence
  Synthetic
DIQMTQSPSSLSASVGDRVTITC

SEQ ID NO: 41 - protein, 22 aa, Artificial Sequence
  Synthetic
QAVVTQEPSLTVSPGGTVTLTC

SEQ ID NO: 42 - protein, 23 aa, Artificial Sequence
  Synthetic
EIVMTQSPATLSVSPGERATLSC

SEQ ID NO: 43 - protein, 23 aa, Artificial Sequence
  Synthetic
EIVMTQSPASLSVSPGERATLSC

SEQ ID NO: 44 - protein, 23 aa, Artificial Sequence
  Synthetic
DIQLTQSPATLSVSPGERATLSC

SEQ ID NO: 45 - protein, 11 aa, Artificial Sequence
  Synthetic
KASQGFNKYVA

SEQ ID NO: 46 - protein, 14 aa, Artificial Sequence
  Synthetic
RSSTGAVTTSNYAN

SEQ ID NO: 47 - protein, 11 aa, Artificial Sequence
  Synthetic
RASQSISSNLG

SEQ ID NO: 48 - protein, 11 aa, Artificial Sequence
  Synthetic
RASQSVSSNLA

SEQ ID NO: 49 - protein, 15 aa, Artificial Sequence
  Synthetic
WYQQKPGKAPKLLIY

SEQ ID NO: 50 - protein, 15 aa, Artificial Sequence
  Synthetic
WVQQKPGQAPRGLIG

SEQ ID NO: 51 - protein, 15 aa, Artificial Sequence
  Synthetic
WYQQKPGQAPRLLIY

SEQ ID NO: 52 - protein, 7 aa, Artificial Sequence
  Synthetic
YTSTLQP

SEQ ID NO: 53 - protein, 7 aa, Artificial Sequence
  Synthetic
GTNKRAP

SEQ ID NO: 54 - protein, 7 aa, Artificial Sequence
  Synthetic
GASTRAT

SEQ ID NO: 55 - protein, 7 aa, Artificial Sequence
  Synthetic
GDYIRAT

SEQ ID NO: 56 - protein, 32 aa, Artificial Sequence
  Synthetic
GVPSRFSGSGSGRDYTLTISSLQPEDFATYYC

SEQ ID NO: 57 - protein, 32 aa, Artificial Sequence
  Synthetic
WTPARFSGSLLGDKAALTLLGAQPEDEAEYFC

SEQ ID NO: 58 - protein, 32 aa, Artificial Sequence
  Synthetic
GIPARFSGSGSGTEFTLTISSLQSEDFAVYYC

SEQ ID NO: 59 - protein, 32 aa, Artificial Sequence
  Synthetic
GIPARVSGGGSGTEFTLTISSLQSEDFAVYCC

SEQ ID NO: 60 - protein, 32 aa, Artificial Sequence
  Synthetic
GIPARFSGSGSGTEFTLTISSLQSEDIATYYC

SEQ ID NO: 61 - protein, 32 aa, Artificial Sequence
  Synthetic
GIPARVSGGGSGTEFTLTISSLQSEDFAVYYC

SEQ ID NO: 62 - protein, 9 aa, Artificial Sequence
  Synthetic
LQYGDLLYA

SEQ ID NO: 63 - protein, 9 aa, Artificial Sequence
  Synthetic
ALWYSNLWV

SEQ ID NO: 64 - protein, 10 aa, Artificial Sequence
  Synthetic
QQYNSWPPLT

SEQ ID NO: 65 - protein, 9 aa, Artificial Sequence
  Synthetic
QQYKNWPFT

SEQ ID NO: 66 - protein, 9 aa, Artificial Sequence
  Synthetic
QQYVDLPIT

SEQ ID NO: 67 - protein, 10 aa, Artificial Sequence
  Synthetic
QQYQSWPPLT

SEQ ID NO: 68 - protein, 9 aa, Artificial Sequence
  Synthetic
QQYHSFPFT

SEQ ID NO: 69 - protein, 10 aa, Artificial Sequence
  Synthetic
QQYRSWPPLT

SEQ ID NO: 70 - protein, 10 aa, Artificial Sequence
  Synthetic
FGQGTKVEIK

SEQ ID NO: 71 - protein, 10 aa, Artificial Sequence
  Synthetic
FGGGTKLTVL

SEQ ID NO: 72 - protein, 10 aa, Artificial Sequence
  Synthetic
FGGGTKVEIK

SEQ ID NO: 73 - protein, 10 aa, Artificial Sequence
  Synthetic
FGPGTKLEIK

SEQ ID NO: 74 - protein, 10 aa, Artificial Sequence
  Synthetic
FGQGTRLEIK

SEQ ID NO: 75 - protein, 121 aa, Artificial Sequence
  Synthetic
EVQLVQSGAEVKKPGASVKVSCKASGYTFTSYWIGWVRQAPGQGLEWIGDIYPGGGYTNYNEKFKGRVTITRDTSTSTAYLELSSLRSEDTAVYYCARLAGSSYRGAMDSWGQGTLVTVSS

SEQ ID NO: 76 - protein, 125 aa, Artificial Sequence
  Synthetic
EVQLVESGGGLVQPGGSLKLSCAASGFTFNTYAMNWVRQASGKGLEWVGRIRSKYNNYATYYADSVKDRFTISRDDSKSTLYLQMNSLKTEDTAVYYCVRHGNFGNSYVSWFAYWGQGTLVTVSS

SEQ ID NO: 77 - protein, 119 aa, Artificial Sequence
  Synthetic
QVQLVESGGGVVQPGRSLRLSCAASGFTFRSFGMHWVRQAPGKGLEWVAVISYDGSNEYYADSVKGRFIISRDNSKDTLYLQMNSLRAGDTAVYYCAKGGGLRWYFAYWGQGTLVTVSS

SEQ ID NO: 78 - protein, 125 aa, Artificial Sequence
  Synthetic
EVQLLESGGGLVQPGGSLRLSCAASGFTFSTYAMNWVRQAPGKGLEWVSRIRSKYNNYATYYADSVKDRFTISRDDSKSTLYLQMNSLRAEDTAVYYCVRHGNFGNSYVSWFAYWGQGTLVTVSS

SEQ ID NO: 79 - protein, 116 aa, Artificial Sequence
  Synthetic
QVQLVQSGAEVKKPGSSMRVSCKASEDTFSSYAISWVRQAPGQGLEWMGGTAPIFGTTNYAQKFQGRVTITADKSTSTAYMELSSLRSEDTAVYYCARGGPYFDYWGQGTLVTVSS

SEQ ID NO: 80 - protein, 119 aa, Artificial Sequence
  Synthetic
QVQLVESGGGVVQPGRSLRLSCAASGFTFRSFGMHWVRQAPGKGLEWVAVISYEGSNEYYADSVKGRFIISRDNSKDTLYLQMNSLRAGDTAVYYCAKGGGLRWYFAYWGQGTLVTVSS

SEQ ID NO: 81 - protein, 119 aa, Artificial Sequence
  Synthetic
QVQLVESGGGVVQPGRSLRLSCAASGFTFRSFGMHWVRQAPGKGLEWVAVISYDASNEYYADSVKGRFIISRDNSKDTLYLQMNSLRAGDTAVYYCAKGGGLRWYFAYWGQGTLVTVSS

SEQ ID NO: 82 - protein, 120 aa, Artificial Sequence
  Synthetic
QLQLQESGPGLVKPSETLSLTCTVSGGSIKSGSYYWGWIRQPPGKGLEWIGNIYYSGSTYYNPSLRSRVTISVDTSKNQFSLKLSSVTAADTAVYYCAREGSYPNQFDPWGQGTLVTVSS

SEQ ID NO: 83 - protein, 119 aa, Artificial Sequence
  Synthetic
QVQLVESGGGVVQPGRSLRLSCAASGFTFRSFGMHWVRQAPGKGLEWVAVISYDASNEYYADSVKGRFIISRDNSKDTLYLQMNSLRAGDTAVYYCAKGGALRWYFAYWGQGTLVTVSS

SEQ ID NO: 84 - protein, 125 aa, Artificial Sequence
  Synthetic
EVQLVESGGGLVQPGGSLKLSCAASGFTFSTYAMNWVRQASGKGLEWVGRIRSKYNNYATYYADSVKDRFTISRDDSKNTAYLQMNSLKTEDTAVYYCTRHGNFGNSYVSWFAYWGQGTLVTVSS

SEQ ID NO: 85 - protein, 107 aa, Artificial Sequence
  Synthetic
DIQMTQSPSSLSASVGDRVTITCKASQGFNKYVAWYQQKPGKAPKLLIYYTSTLQPGVPSRFSGSGSGRDYTLTISSLQPEDFATYYCLQYGDLLYAFGQGTKVEIK

SEQ ID NO: 86 - protein, 109 aa, Artificial Sequence
  Synthetic
QAVVTQEPSLTVSPGGTVTLTCRSSTGAVTTSNYANWVQQKPGQAPRGLIGGTNKRAPWTPARFSGSLLGDKAALTLLGAQPEDEAEYFCALWYSNLWVFGGGTKLTVL

SEQ ID NO: 87 - protein, 108 aa, Artificial Sequence
  Synthetic
EIVMTQSPATLSVSPGERATLSCRASQSISSNLGWYQQKPGQAPRLLIYGASTRATGIPARFSGSGSGTEFTLTISSLQSEDFAVYYCQQYNSWPPLTFGGGTKVEIK

SEQ ID NO: 88 - protein, 107 aa, Artificial Sequence
  Synthetic
EIVMTQSPASLSVSPGERATLSCRASQSVSSNLAWYQQKPGQAPRLLIYGASTRATGIPARVSGGGSGTEFTLTISSLQSEDFAVYCCQQYKNWPFTFGPGTKLEIK

SEQ ID NO: 89 - protein, 107 aa, Artificial Sequence
  Synthetic
DIQLTQSPATLSVSPGERATLSCRASQSVSSNLAWYQQKPGQAPRLLIYGDYIRATGIPARFSGSGSGTEFTLTISSLQSEDIATYYCQQYVDLPITFGQGTRLEIK

SEQ ID NO: 90 - protein, 108 aa, Artificial Sequence
  Synthetic
EIVMTQSPATLSVSPGERATLSCRASQSISSNLGWYQQKPGQAPRLLIYGASTRATGIPARFSGSGSGTEFTLTISSLQSEDFAVYYCQQYQSWPPLTFGGGTKVEIK

SEQ ID NO: 91 - protein, 107 aa, Artificial Sequence
  Synthetic
EIVMTQSPASLSVSPGERATLSCRASQSVSSNLAWYQQKPGQAPRLLIYGASTRATGIPARVSGGGSGTEFTLTISSLQSEDFAVYYCQQYKNWPFTFGPGTKLEIK

SEQ ID NO: 92 - protein, 107 aa, Artificial Sequence
  Synthetic
EIVMTQSPATLSVSPGERATLSCRASQSVSSNLAWYQQKPGQAPRLLIYGASTRATGIPARFSGSGSGTEFTLTISSLQSEDFAVYYCQQYHSFPFTFGGGTKVEIK

SEQ ID NO: 93 - protein, 108 aa, Artificial Sequence
  Synthetic
EIVMTQSPATLSVSPGERATLSCRASQSISSNLGWYQQKPGQAPRLLIYGASTRATGIPARFSGSGSGTEFTLTISSLQSEDFAVYYCQQYRSWPPLTFGGGTKVEIK

SEQ ID NO: 94 - protein, 451 aa, Artificial Sequence
  Synthetic
EVQLVQSGAEVKKPGASVKVSCKASGYTFTSYWIGWVRQAPGQGLEWIGDIYPGGGYTNYNEKFKGRVTITRDTSTSTAYLELSSLRSEDTAVYYCARLAGSSYRGAMDSWGQGTLVTVSSASTKGPSVFPLAPSSKSTSGGTAALGCLVKDYFPEPVTVSWNSGALTSGVHTFPAVLQSSGLYSLSSVVTVPSSSLGTQTYICNVNHKPSNTKVDKKVEPKSCDKTHTCPPCPAPELLGGPSVFLFPPKPKDTLMISRTPEVTCVVVDVSHEDPEVKFNWYVDGVEVHNAKTKPREEQYNSTYRVVSVLTVLHQDWLNGKEYKCKVSNKALPAPIEKTISKAKGQPREPQVYTLPPSREEMTKNQVSLTCLVKGFYPSDIAVEWESNGQPENNYKTTPPVLDSDGSFFLYSKLTVDKSRWQQGNVFSCSVMHEALHNHYTQKSLSLSPGK

SEQ ID NO: 95 - protein, 449 aa, Artificial Sequence
  Synthetic
QVQLVESGGGVVQPGRSLRLSCAASGFTFRSFGMHWVRQAPGKGLEWVAVISYDGSNEYYADSVKGRFIISRDNSKDTLYLQMNSLRAGDTAVYYCAKGGGLRWYFAYWGQGTLVTVSSASTKGPSVFPLAPSSKSTSGGTAALGCLVKDYFPEPVTVSWNSGALTSGVHTFPAVLQSSGLYSLSSVVTVPSSSLGTQTYICNVNHKPSNTKVDKKVEPKSCDKTHTCPPCPAPELLGGPSVFLFPPKPKDTLMISRTPEVTCVVVDVSHEDPEVKFNWYVDGVEVHNAKTKPREEQYNSTYRVVSVLTVLHQDWLNGKEYKCKVSNKALPAPIEKTISKAKGQPREPQVYTLPPSREEMTKNQVSLTCLVKGFYPSDIAVEWESNGQPENNYKTTPPVLDSDGSFFLYSKLTVDKSRWQQGNVFSCSVMHEALHNHYTQKSLSLSPGK

SEQ ID NO: 96 - protein, 455 aa, Artificial Sequence
  Synthetic
EVQLLESGGGLVQPGGSLRLSCAASGFTFSTYAMNWVRQAPGKGLEWVSRIRSKYNNYATYYADSVKDRFTISRDDSKSTLYLQMNSLRAEDTAVYYCVRHGNFGNSYVSWFAYWGQGTLVTVSSASTKGPSVFPLAPSSKSTSGGTAALGCLVKDYFPEPVTVSWNSGALTSGVHTFPAVLQSSGLYSLSSVVTVPSSSLGTQTYICNVNHKPSNTKVDKKVEPKSCDKTHTCPPCPAPEAAGGPSVFLFPPKPKDTLMISRTPEVTCVVVDVSHEDPEVKFNWYVDGVEVHNAKTKPREEQYNSTYRVVSVLTVLHQDWLNGKEYKCKVSNKALGAPIEKTISKAKGQPREPQVYTLPPSREEMTKNQVSLTCLVKGFYPSDIAVEWESNGQPENNYKTTPPVLDSDGSFFLYSKLTVDKSRWQQGNVFSCSVMHEALHNHYTQKSLSLSPGK

SEQ ID NO: 97 - protein, 228 aa, Artificial Sequence
  Synthetic
EVQLLESGGGLVQPGGSLRLSCAASGFTFSTYAMNWVRQAPGKGLEWVSRIRSKYNNYATYYADSVKDRFTISRDDSKSTLYLQMNSLRAEDTAVYYCVRHGNFGNSYVSWFAYWGQGTLVTVSSASTKGPSVFPLAPSSKSTSGGTAALGCLVKDYFPEPVTVSWNSGALTSGVHTFPAVLQSSGLYSLSSVVTVPSSSLGTQTYICNVNHKPSNTKVDKKVEPKSC

SEQ ID NO: 98 - protein, 446 aa, Artificial Sequence
  Synthetic
QVQLVQSGAEVKKPGSSMRVSCKASEDTFSSYAISWVRQAPGQGLEWMGGTAPIFGTTNYAQKFQGRVTITADKSTSTAYMELSSLRSEDTAVYYCARGGPYFDYWGQGTLVTVSSASTKGPSVFPLAPSSKSTSGGTAALGCLVKDYFPEPVTVSWNSGALTSGVHTFPAVLQSSGLYSLSSVVTVPSSSLGTQTYICNVNHKPSNTKVDKKVEPKSCDKTHTCPPCPAPELLGGPSVFLFPPKPKDTLMISRTPEVTCVVVDVSHEDPEVKFNWYVDGVEVHNAKTKPREEQYNSTYRVVSVLTVLHQDWLNGKEYKCKVSNKALPAPIEKTISKAKGQPREPQVYTLPPSREEMTKNQVSLTCLVKGFYPSDIAVEWESNGQPENNYKTTPPVLDSDGSFFLYSKLTVDKSRWQQGNVFSCSVMHEALHNHYTQKSLSLSPGK

SEQ ID NO: 99 - protein, 449 aa, Artificial Sequence
  Synthetic
QVQLVESGGGVVQPGRSLRLSCAASGFTFRSFGMHWVRQAPGKGLEWVAVISYEGSNEYYADSVKGRFIISRDNSKDTLYLQMNSLRAGDTAVYYCAKGGGLRWYFAYWGQGTLVTVSSASTKGPSVFPLAPSSKSTSGGTAALGCLVKDYFPEPVTVSWNSGALTSGVHTFPAVLQSSGLYSLSSVVTVPSSSLGTQTYICNVNHKPSNTKVDKKVEPKSCDKTHTCPPCPAPELLGGPSVFLFPPKPKDTLMISRTPEVTCVVVDVSHEDPEVKFNWYVDGVEVHNAKTKPREEQYNSTYRVVSVLTVLHQDWLNGKEYKCKVSNKALPAPIEKTISKAKGQPREPQVYTLPPSREEMTKNQVSLTCLVKGFYPSDIAVEWESNGQPENNYKTTPPVLDSDGSFFLYSKLTVDKSRWQQGNVFSCSVMHEALHNHYTQKSLSLSPGK

SEQ ID NO: 100 - protein, 449 aa, Artificial Sequence
  Synthetic
QVQLVESGGGVVQPGRSLRLSCAASGFTFRSFGMHWVRQAPGKGLEWVAVISYDASNEYYADSVKGRFIISRDNSKDTLYLQMNSLRAGDTAVYYCAKGGGLRWYFAYWGQGTLVTVSSASTKGPSVFPLAPSSKSTSGGTAALGCLVKDYFPEPVTVSWNSGALTSGVHTFPAVLQSSGLYSLSSVVTVPSSSLGTQTYICNVNHKPSNTKVDKKVEPKSCDKTHTCPPCPAPELLGGPSVFLFPPKPKDTLMISRTPEVTCVVVDVSHEDPEVKFNWYVDGVEVHNAKTKPREEQYNSTYRVVSVLTVLHQDWLNGKEYKCKVSNKALPAPIEKTISKAKGQPREPQVYTLPPSREEMTKNQVSLTCLVKGFYPSDIAVEWESNGQPENNYKTTPPVLDSDGSFFLYSKLTVDKSRWQQGNVFSCSVMHEALHNHYTQKSLSLSPGK

SEQ ID NO: 101 - protein, 449 aa, Artificial Sequence
  Synthetic
QVQLVESGGGVVQPGRSLRLSCAASGFTFRSFGMHWVRQAPGKGLEWVAVISYDGSNEYYADSVKGRFIISRDNSKDTLYLQMNSLRAGDTAVYYCAKGGGLRWYFAYWGQGTLVTVSSASTKGPSVFPLAPSSKSTSGGTAALGCLVKDYFPEPVTVSWNSGALTSGVHTFPAVLQSSGLYSLSSVVTVPSSSLGTQTYICNVNHKPSNTKVDKKVEPKSCDKTHTCPPCPAPELLGGPDVFLFPPKPKDTLMISRTPEVTCVVVDVSHEDPEVKFNWYVDGVEVHNAKTKPREEQYNSTYRVVSVLTVLHQDWLNGKEYKCKVSNKALPAPEEKTISKAKGQPREPQVYTLPPSREEMTKNQVSLTCLVKGFYPSDIAVEWESNGQPENNYKTTPPVLDSDGSFFLYSKLTVDKSRWQQGNVFSCSVMHEALHNHYTQKSLSLSPGK

SEQ ID NO: 102 - protein, 449 aa, Artificial Sequence
  Synthetic
QVQLVESGGGVVQPGRSLRLSCAASGFTFRSFGMHWVRQAPGKGLEWVAVISYDASNEYYADSVKGRFIISRDNSKDTLYLQMNSLRAGDTAVYYCAKGGGLRWYFAYWGQGTLVTVSSASTKGPSVFPLAPSSKSTSGGTAALGCLVKDYFPEPVTVSWNSGALTSGVHTFPAVLQSSGLYSLSSVVTVPSSSLGTQTYICNVNHKPSNTKVDKKVEPKSCDKTHTCPPCPAPELLGGPDVFLFPPKPKDTLMISRTPEVTCVVVDVSHEDPEVKFNWYVDGVEVHNAKTKPREEQYNSTYRVVSVLTVLHQDWLNGKEYKCKVSNKALPAPEEKTISKAKGQPREPQVYTLPPSREEMTKNQVSLTCLVKGFYPSDIAVEWESNGQPENNYKTTPPVLDSDGSFFLYSKLTVDKSRWQQGNVFSCSVMHEALHNHYTQKSLSLSPGK

SEQ ID NO: 103 - protein, 446 aa, Artificial Sequence
  Synthetic
QVQLVQSGAEVKKPGSSMRVSCKASEDTFSSYAISWVRQAPGQGLEWMGGTAPIFGTTNYAQKFQGRVTITADKSTSTAYMELSSLRSEDTAVYYCARGGPYFDYWGQGTLVTVSSASTKGPSVFPLAPSSKSTSGGTAALGCLVKDYFPEPVTVSWNSGALTSGVHTFPAVLQSSGLYSLSSVVTVPSSSLGTQTYICNVNHKPSNTKVDKKVEPKSCDKTHTCPPCPAPELLGGPDVFLFPPKPKDTLMISRTPEVTCVVVDVSHEDPEVKFNWYVDGVEVHNAKTKPREEQYNSTYRVVSVLTVLHQDWLNGKEYKCKVSNKALPAPEEKTISKAKGQPREPQVYTLPPSREEMTKNQVSLTCLVKGFYPSDIAVEWESNGQPENNYKTTPPVLDSDGSFFLYSKLTVDKSRWQQGNVFSCSVMHEALHNHYTQKSLSLSPGK

SEQ ID NO: 104 - protein, 450 aa, Artificial Sequence
  Synthetic
QLQLQESGPGLVKPSETLSLTCTVSGGSIKSGSYYWGWIRQPPGKGLEWIGNIYYSGSTYYNPSLRSRVTISVDTSKNQFSLKLSSVTAADTAVYYCAREGSYPNQFDPWGQGTLVTVSSASTKGPSVFPLAPSSKSTSGGTAALGCLVKDYFPEPVTVSWNSGALTSGVHTFPAVLQSSGLYSLSSVVTVPSSSLGTQTYICNVNHKPSNTKVDKKVEPKSCDKTHTCPPCPAPELLGGPSVFLFPPKPKDTLMISRTPEVTCVVVDVSHEDPEVKFNWYVDGVEVHNAKTKPREEQYNSTYRVVSVLTVLHQDWLNGKEYKCKVSNKALPAPIEKTISKAKGQPREPQVYTLPPSREEMTKNQVSLTCLVKGFYPSDIAVEWESNGQPENNYKTTPPVLDSDGSFFLYSKLTVDKSRWQQGNVFSCSVMHEALHNHYTQKSLSLSPGK

SEQ ID NO: 105 - protein, 450 aa, Artificial Sequence
  Synthetic
QLQLQESGPGLVKPSETLSLTCTVSGGSIKSGSYYWGWIRQPPGKGLEWIGNIYYSGSTYYNPSLRSRVTISVDTSKNQFSLKLSSVTAADTAVYYCAREGSYPNQFDPWGQGTLVTVSSASTKGPSVFPLAPSSKSTSGGTAALGCLVKDYFPEPVTVSWNSGALTSGVHTFPAVLQSSGLYSLSSVVTVPSSSLGTQTYICNVNHKPSNTKVDKKVEPKSCDKTHTCPPCPAPELLGGPDVFLFPPKPKDTLMISRTPEVTCVVVDVSHEDPEVKFNWYVDGVEVHNAKTKPREEQYNSTYRVVSVLTVLHQDWLNGKEYKCKVSNKALPAPEEKTISKAKGQPREPQVYTLPPSREEMTKNQVSLTCLVKGFYPSDIAVEWESNGQPENNYKTTPPVLDSDGSFFLYSKLTVDKSRWQQGNVFSCSVMHEALHNHYTQKSLSLSPGK

SEQ ID NO: 106 - protein, 449 aa, Artificial Sequence
  Synthetic
QVQLVESGGGVVQPGRSLRLSCAASGFTFRSFGMHWVRQAPGKGLEWVAVISYDASNEYYADSVKGRFIISRDNSKDTLYLQMNSLRAGDTAVYYCAKGGALRWYFAYWGQGTLVTVSSASTKGPSVFPLAPSSKSTSGGTAALGCLVKDYFPEPVTVSWNSGALTSGVHTFPAVLQSSGLYSLSSVVTVPSSSLGTQTYICNVNHKPSNTKVDKKVEPKSCDKTHTCPPCPAPELLGGPDVFLFPPKPKDTLMISRTPEVTCVVVDVSHEDPEVKFNWYVDGVEVHNAKTKPREEQYNSTYRVVSVLTVLHQDWLNGKEYKCKVSNKALPAPEEKTISKAKGQPREPQVYTLPPSREEMTKNQVSLTCLVKGFYPSDIAVEWESNGQPENNYKTTPPVLDSDGSFFLYSKLTVDKSRWQQGNVFSCSVMHEALHNHYTQKSLSLSPGK

SEQ ID NO: 107 - protein, 455 aa, Artificial Sequence
  Synthetic
EVQLVESGGGLVQPGGSLKLSCAASGFTFSTYAMNWVRQASGKGLEWVGRIRSKYNNYATYYADSVKDRFTISRDDSKNTAYLQMNSLKTEDTAVYYCTRHGNFGNSYVSWFAYWGQGTLVTVSSASTKGPSVFPLAPSSKSTSGGTAALGCLVKDYFPEPVTVSWNSGALTSGVHTFPAVLQSSGLYSLSSVVTVPSSSLGTQTYICNVNHKPSNTKVDKKVEPKSCDKTHTCPPCPAPEAAGGPSVFLFPPKPKDTLMISRTPEVTCVVVDVSHEDPEVKFNWYVDGVEVHNAKTKPREEQYNSTYRVVSVLTVLHQDWLNGKEYKCKVSNKALPAPIEKTISKAKGQPREPQVYTLPPSREEMTKNQVSLTCLVKGFYPSDIAVEWESNGQPENNYKTTPPVLDSDGSFFLYSKLTVDKSRWQQGNVFSCSVMHEALHNHYTQKSLSLSPGK

SEQ ID NO: 108 - protein, 214 aa, Artificial Sequence
  Synthetic
DIQMTQSPSSLSASVGDRVTITCKASQGFNKYVAWYQQKPGKAPKLLIYYTSTLQPGVPSRFSGSGSGRDYTLTISSLQPEDFATYYCLQYGDLLYAFGQGTKVEIKRTVAAPSVFIFPPSDEQLKSGTASVVCLLNNFYPREAKVQWKVDNALQSGNSQESVTEQDSKDSTYSLSSTLTLSKADYEKHKVYACEVTHQGLSSPVTKSFNRGEC

SEQ ID NO: 109 - protein, 215 aa, Artificial Sequence
  Synthetic
EIVMTQSPATLSVSPGERATLSCRASQSISSNLGWYQQKPGQAPRLLIYGASTRATGIPARFSGSGSGTEFTLTISSLQSEDFAVYYCQQYNSWPPLTFGGGTKVEIKRTVAAPSVFIFPPSDEQLKSGTASVVCLLNNFYPREAKVQWKVDNALQSGNSQESVTEQDSKDSTYSLSSTLTLSKADYEKHKVYACEVTHQGLSSPVTKSFNRGEC

SEQ ID NO: 110 - protein, 215 aa, Artificial Sequence
  Synthetic
QAVVTQEPSLTVSPGGTVTLTCRSSTGAVTTSNYANWVQQKPGQAPRGLIGGTNKRAPWTPARFSGSLLGDKAALTLLGAQPEDEAEYFCALWYSNLWVFGGGTKLTVLGQPKAAPSVTLFPPSSEELQANKATLVCLISDFYPGAVTVAWKADSSPVKAGVETTTPSKQSNNKYAASSYLSLTPEQWKSHRSYSCQVTHEGSTVEKTVAPTECS

SEQ ID NO: 111 - protein, 442 aa, Artificial Sequence
  Synthetic
QAVVTQEPSLTVSPGGTVTLTCRSSTGAVTTSNYANWVQQKPGQAPRGLIGGTNKRAPWTPARFSGSLLGDKAALTLLGAQPEDEAEYFCALWYSNLWVFGGGTKLTVLGQPKAAPSVTLFPPSSEELQANKATLVCLISDFYPGAVTVAWKADSSPVKAGVETTTPSKQSNNKYAASSYLSLTPEQWKSHRSYSCQVTHEGSTVEKTVAPTECSDKTHTCPPCPAPEAAGGPSVFLFPPKPKDTLMISRTPEVTCVVVDVSHEDPEVKFNWYVDGVEVHNAKTKPREEQYNSTYRVVSVLTVLHQDWLNGKEYKCKVSNKALGAPIEKTISKAKGQPREPQVYTLPPSREEMTKNQVSLTCLVKGFYPSDIAVEWESNGQPENNYKTTPPVLDSDGSFFLYSKLTVDKSRWQQGNVFSCSVMHEALHNHYTQKSLSLSPGK

SEQ ID NO: 112 - protein, 214 aa, Artificial Sequence
  Synthetic
EIVMTQSPASLSVSPGERATLSCRASQSVSSNLAWYQQKPGQAPRLLIYGASTRATGIPARVSGGGSGTEFTLTISSLQSEDFAVYCCQQYKNWPFTFGPGTKLEIKRTVAAPSVFIFPPSDEQLKSGTASVVCLLNNFYPREAKVQWKVDNALQSGNSQESVTEQDSKDSTYSLSSTLTLSKADYEKHKVYACEVTHQGLSSPVTKSFNRGEC

SEQ ID NO: 113 - protein, 214 aa, Artificial Sequence
  Synthetic
DIQLTQSPATLSVSPGERATLSCRASQSVSSNLAWYQQKPGQAPRLLIYGDYIRATGIPARFSGSGSGTEFTLTISSLQSEDIATYYCQQYVDLPITFGQGTRLEIKRTVAAPSVFIFPPSDEQLKSGTASVVCLLNNFYPREAKVQWKVDNALQSGNSQESVTEQDSKDSTYSLSSTLTLSKADYEKHKVYACEVTHQGLSSPVTKSFNRGEC

SEQ ID NO: 114 - protein, 215 aa, Artificial Sequence
  Synthetic
EIVMTQSPATLSVSPGERATLSCRASQSISSNLGWYQQKPGQAPRLLIYGASTRATGIPARFSGSGSGTEFTLTISSLQSEDFAVYYCQQYQSWPPLTFGGGTKVEIKRTVAAPSVFIFPPSDEQLKSGTASVVCLLNNFYPREAKVQWKVDNALQSGNSQESVTEQDSKDSTYSLSSTLTLSKADYEKHKVYACEVTHQGLSSPVTKSFNRGEC

SEQ ID NO: 115 - protein, 214 aa, Artificial Sequence
  Synthetic
EIVMTQSPASLSVSPGERATLSCRASQSVSSNLAWYQQKPGQAPRLLIYGASTRATGIPARVSGGGSGTEFTLTISSLQSEDFAVYYCQQYKNWPFTFGPGTKLEIKRTVAAPSVFIFPPSDEQLKSGTASVVCLLNNFYPREAKVQWKVDNALQSGNSQESVTEQDSKDSTYSLSSTLTLSKADYEKHKVYACEVTHQGLSSPVTKSFNRGEC

SEQ ID NO: 116 - protein, 214 aa, Artificial Sequence
  Synthetic
EIVMTQSPATLSVSPGERATLSCRASQSVSSNLAWYQQKPGQAPRLLIYGASTRATGIPARFSGSGSGTEFTLTISSLQSEDFAVYYCQQYHSFPFTFGGGTKVEIKRTVAAPSVFIFPPSDEQLKSGTASVVCLLNNFYPREAKVQWKVDNALQSGNSQESVTEQDSKDSTYSLSSTLTLSKADYEKHKVYACEVTHQGLSSPVTKSFNRGEC

SEQ ID NO: 117 - protein, 215 aa, Artificial Sequence
  Synthetic
EIVMTQSPATLSVSPGERATLSCRASQSISSNLGWYQQKPGQAPRLLIYGASTRATGIPARFSGSGSGTEFTLTISSLQSEDFAVYYCQQYRSWPPLTFGGGTKVEIKRTVAAPSVFIFPPSDEQLKSGTASVVCLLNNFYPREAKVQWKVDNALQSGNSQESVTEQDSKDSTYSLSSTLTLSKADYEKHKVYACEVTHQGLSSPVTKSFNRGEC

SEQ ID NO: 118 - protein, 449 aa, Artificial Sequence
  Synthetic
QVQLVESGGGVVQPGRSLRLSCAASGFTFRSFGMHWVRQAPGKGLEWVAVISYDGSNEYYADSVKGRFIISRDNSKDTLYLQMNSLRAGDTAVYYCAKGGGLRWYFAYWGQGTLVTVSSASTKGPSVFPLAPSSKSTSGGTAALGCLVKDYFPEPVTVSWNSGALTSGVHTFPAVLQSSGLYSLSSVVTVPSSSLGTQTYICNVNHKPSNTKVDKKVEPKSCDKTHTCPPCPAPEAAGGPSVFLFPPKPKDTLMISRTPEVTCVVVDVSHEDPEVKFNWYVDGVEVHNAKTKPREEQYNSTYRVVSVLTVLHQDWLNGKEYKCKVSNKALGAPIEKTISKAKGQPREPQVCTLPPSREEMTKNQVSLSCAVKGFYPSDIAVEWESNGQPENNYKTTPPVLDSDGSFFLVSKLTVDKSRWQQGNVFSCSVMHEALHNHYTQKSLSLSPGK

SEQ ID NO: 119 - protein, 483 aa, Artificial Sequence
  Synthetic
QAVVTQEPSLTVSPGGTVTLTCRSSTGAVTTSNYANWVQQKPGQAPRGLIGGTNKRAPWTPARFSGSLLGDKAALTLLGAQPEDEAEYFCALWYSNLWVFGGGTKLTVLGGGQSGQGGSGGGGSEVQLVESGGGLVQPGGSLKLSCAASGFTFNTYAMNWVRQASGKGLEWVGRIRSKYNNYATYYADSVKDRFTISRDDSKSTLYLQMNSLKTEDTAVYYCVRHGNFGNSYVSWFAYWGQGTLVTVSSASEPKSSDKTHTCPPCPAPEAAGGPSVFLFPPKPKDTLMISRTPEVTCVVVDVSHEDPEVKFNWYVDGVEVHNAKTKPREEQYNSTYRVVSVLTVLHQDWLNGKEYKCKVSNKALGAPIEKTISKAKGQPREPQVYTLPPCREEMTKNQVSLWCLVKGFYPSDIAVEWESNGQPENNYKTTPPVLDSDGSFFLYSKLTVDKSRWQQGNVFSCSVMHEALHNHYTQKSLSLSPGK

SEQ ID NO: 120 - protein, 449 aa, Artificial Sequence
  Synthetic
QVQLVESGGGVVQPGRSLRLSCAASGFTFRSFGMHWVRQAPGKGLEWVAVISYEGSNEYYADSVKGRFIISRDNSKDTLYLQMNSLRAGDTAVYYCAKGGGLRWYFAYWGQGTLVTVSSASTKGPSVFPLAPSSKSTSGGTAALGCLVKDYFPEPVTVSWNSGALTSGVHTFPAVLQSSGLYSLSSVVTVPSSSLGTQTYICNVNHKPSNTKVDKKVEPKSCDKTHTCPPCPAPEAAGGPSVFLFPPKPKDTLMISRTPEVTCVVVDVSHEDPEVKFNWYVDGVEVHNAKTKPREEQYNSTYRVVSVLTVLHQDWLNGKEYKCKVSNKALGAPIEKTISKAKGQPREPQVCTLPPSREEMTKNQVSLSCAVKGFYPSDIAVEWESNGQPENNYKTTPPVLDSDGSFFLVSKLTVDKSRWQQGNVFSCSVMHEALHNHYTQKSLSLSPGK

SEQ ID NO: 121 - protein, 449 aa, Artificial Sequence
  Synthetic
QVQLVESGGGVVQPGRSLRLSCAASGFTFRSFGMHWVRQAPGKGLEWVAVISYDASNEYYADSVKGRFIISRDNSKDTLYLQMNSLRAGDTAVYYCAKGGGLRWYFAYWGQGTLVTVSSASTKGPSVFPLAPSSKSTSGGTAALGCLVKDYFPEPVTVSWNSGALTSGVHTFPAVLQSSGLYSLSSVVTVPSSSLGTQTYICNVNHKPSNTKVDKKVEPKSCDKTHTCPPCPAPEAAGGPSVFLFPPKPKDTLMISRTPEVTCVVVDVSHEDPEVKFNWYVDGVEVHNAKTKPREEQYNSTYRVVSVLTVLHQDWLNGKEYKCKVSNKALGAPIEKTISKAKGQPREPQVCTLPPSREEMTKNQVSLSCAVKGFYPSDIAVEWESNGQPENNYKTTPPVLDSDGSFFLVSKLTVDKSRWQQGNVFSCSVMHEALHNHYTQKSLSLSPGK

SEQ ID NO: 122 - protein, 446 aa, Artificial Sequence
  Synthetic
QVQLVQSGAEVKKPGSSMRVSCKASEDTFSSYAISWVRQAPGQGLEWMGGTAPIFGTTNYAQKFQGRVTITADKSTSTAYMELSSLRSEDTAVYYCARGGPYFDYWGQGTLVTVSSASTKGPSVFPLAPSSKSTSGGTAALGCLVKDYFPEPVTVSWNSGALTSGVHTFPAVLQSSGLYSLSSVVTVPSSSLGTQTYICNVNHKPSNTKVDKKVEPKSCDKTHTCPPCPAPEAAGGPSVFLFPPKPKDTLMISRTPEVTCVVVDVSHEDPEVKFNWYVDGVEVHNAKTKPREEQYNSTYRVVSVLTVLHQDWLNGKEYKCKVSNKALGAPIEKTISKAKGQPREPQVCTLPPSREEMTKNQVSLSCAVKGFYPSDIAVEWESNGQPENNYKTTPPVLDSDGSFFLVSKLTVDKSRWQQGNVFSCSVMHEALHNHYTQKSLSLSPGK

SEQ ID NO: 123 - protein, 442 aa, Artificial Sequence
  Synthetic
QAVVTQEPSLTVSPGGTVTLTCRSSTGAVTTSNYANWVQQKPGQAPRGLIGGTNKRAPWTPARFSGSLLGDKAALTLLGAQPEDEAEYFCALWYSNLWVFGGGTKLTVLGQPKAAPSVTLFPPSSEELQANKATLVCLISDFYPGAVTVAWKADSSPVKAGVETTTPSKQSNNKYAASSYLSLTPEQWKSHRSYSCQVTHEGSTVEKTVAPTECSDKTHTCPPCPAPEAAGGPSVFLFPPKPKDTLMISRTPEVTCVVVDVSHEDPEVKFNWYVDGVEVHNAKTKPREEQYNSTYRVVSVLTVLHQDWLNGKEYKCKVSNKALGAPIEKTISKAKGQPREPQVYTLPPCREEMTKNQVSLWCLVKGFYPSDIAVEWESNGQPENNYKTTPPVLDSDGSFFLYSKLTVDKSRWQQGNVFSCSVMHEALHNHYTQKSLSLSPGK

SEQ ID NO: 124 - protein, 669 aa, Artificial Sequence
  Synthetic
QVQLVESGGGVVQPGRSLRLSCAASGFTFRSFGMHWVRQAPGKGLEWVAVISYDGSNEYYADSVKGRFIISRDNSKDTLYLQMNSLRAGDTAVYYCAKGGGLRWYFAYWGQGTLVTVSSASTKGPSVFPLAPSSKSTSGGTAALGCLVKDYFPEPVTVSWNSGALTSGVHTFPAVLQSSGLYSLSSVVTVPSSSLGTQTYICNVNHKPSNTKVDKKVEPKSCGGGGSQAVVTQEPSLTVSPGGTVTLTCRSSTGAVTTSNYANWVQQKPGQAPRGLIGGTNKRAPWTPARFSGSLLGDKAALTLLGAQPEDEAEYFCALWYSNLWVFGGGTKLTVLGQPKAAPSVTLFPPSSEELQANKATLVCLISDFYPGAVTVAWKADSSPVKAGVETTTPSKQSNNKYAASSYLSLTPEQWKSHRSYSCQVTHEGSTVEKTVAPTECSDKTHTCPPCPAPEAAGGPSVFLFPPKPKDTLMISRTPEVTCVVVDVSHEDPEVKFNWYVDGVEVHNAKTKPREEQYNSTYRVVSVLTVLHQDWLNGKEYKCKVSNKALGAPIEKTISKAKGQPREPQVYTLPPCREEMTKNQVSLWCLVKGFYPSDIAVEWESNGQPENNYKTTPPVLDSDGSFFLYSKLTVDKSRWQQGNVFSCSVMHEALHNHYTQKSLSLSPGK

SEQ ID NO: 125 - protein, 668 aa, Artificial Sequence
  Synthetic
QVQLVESGGGVVQPGRSLRLSCAASGFTFRSFGMHWVRQAPGKGLEWVAVISYDGSNEYYADSVKGRFIISRDNSKDTLYLQMNSLRAGDTAVYYCAKGGGLRWYFAYWGQGTLVTVSSASTKGPSVFPLAPSSKSTSGGTAALGCLVKDYFPEPVTVSWNSGALTSGVHTFPAVLQSSGLYSLSSVVTVPSSSLGTQTYICNVNHKPSNTKVDKKVEPKSCDKTHTCPPCPAPEAAGGPSVFLFPPKPKDTLMISRTPEVTCVVVDVSHEDPEVKFNWYVDGVEVHNAKTKPREEQYNSTYRVVSVLTVLHQDWLNGKEYKCKVSNKALGAPIEKTISKAKGQPREPQVYTLPPCREEMTKNQVSLWCLVKGFYPSDIAVEWESNGQPENNYKTTPPVLDSDGSFFLYSKLTVDKSRWQQGNVFSCSVMHEALHNHYTQKSLSLSPGGGGGSQAVVTQEPSLTVSPGGTVTLTCRSSTGAVTTSNYANWVQQKPGQAPRGLIGGTNKRAPWTPARFSGSLLGDKAALTLLGAQPEDEAEYFCALWYSNLWVFGGGTKLTVLGQPKAAPSVTLFPPSSEELQANKATLVCLISDFYPGAVTVAWKADSSPVKAGVETTTPSKQSNNKYAASSYLSLTPEQWKSHRSYSCQVTHEGSTVEKTVAPTECS

SEQ ID NO: 126 - protein, 710 aa, Artificial Sequence
  Synthetic
QVQLVESGGGVVQPGRSLRLSCAASGFTFRSFGMHWVRQAPGKGLEWVAVISYDGSNEYYADSVKGRFIISRDNSKDTLYLQMNSLRAGDTAVYYCAKGGGLRWYFAYWGQGTLVTVSSASTKGPSVFPLAPSSKSTSGGTAALGCLVKDYFPEPVTVSWNSGALTSGVHTFPAVLQSSGLYSLSSVVTVPSSSLGTQTYICNVNHKPSNTKVDKKVEPKSCGGGGSQAVVTQEPSLTVSPGGTVTLTCRSSTGAVTTSNYANWVQQKPGQAPRGLIGGTNKRAPWTPARFSGSLLGDKAALTLLGAQPEDEAEYFCALWYSNLWVFGGGTKLTVLGGGQSGQGGSGGGGSEVQLVESGGGLVQPGGSLKLSCAASGFTFNTYAMNWVRQASGKGLEWVGRIRSKYNNYATYYADSVKDRFTISRDDSKSTLYLQMNSLKTEDTAVYYCVRHGNFGNSYVSWFAYWGQGTLVTVSSASEPKSSDKTHTCPPCPAPEAAGGPSVFLFPPKPKDTLMISRTPEVTCVVVDVSHEDPEVKFNWYVDGVEVHNAKTKPREEQYNSTYRVVSVLTVLHQDWLNGKEYKCKVSNKALGAPIEKTISKAKGQPREPQVYTLPPCREEMTKNQVSLWCLVKGFYPSDIAVEWESNGQPENNYKTTPPVLDSDGSFFLYSKLTVDKSRWQQGNVFSCSVMHEALHNHYTQKSLSLSPGK

SEQ ID NO: 127 - protein, 702 aa, Artificial Sequence
  Synthetic
QVQLVESGGGVVQPGRSLRLSCAASGFTFRSFGMHWVRQAPGKGLEWVAVISYDGSNEYYADSVKGRFIISRDNSKDTLYLQMNSLRAGDTAVYYCAKGGGLRWYFAYWGQGTLVTVSSASTKGPSVFPLAPSSKSTSGGTAALGCLVKDYFPEPVTVSWNSGALTSGVHTFPAVLQSSGLYSLSSVVTVPSSSLGTQTYICNVNHKPSNTKVDKKVEPKSCDKTHTCPPCPAPEAAGGPSVFLFPPKPKDTLMISRTPEVTCVVVDVSHEDPEVKFNWYVDGVEVHNAKTKPREEQYNSTYRVVSVLTVLHQDWLNGKEYKCKVSNKALGAPIEKTISKAKGQPREPQVYTLPPCREEMTKNQVSLWCLVKGFYPSDIAVEWESNGQPENNYKTTPPVLDSDGSFFLYSKLTVDKSRWQQGNVFSCSVMHEALHNHYTQKSLSLSPGGGGGSQAVVTQEPSLTVSPGGTVTLTCRSSTGAVTTSNYANWVQQKPGQAPRGLIGGTNKRAPWTPARFSGSLLGDKAALTLLGAQPEDEAEYFCALWYSNLWVFGGGTKLTVLGGGQSGQGGSGGGGSEVQLVESGGGLVQPGGSLKLSCAASGFTFNTYAMNWVRQASGKGLEWVGRIRSKYNNYATYYADSVKDRFTISRDDSKSTLYLQMNSLKTEDTAVYYCVRHGNFGNSYVSWFAYWGQGTLVTVSS

SEQ ID NO: 128 - protein, 455 aa, Artificial Sequence
  Synthetic
EVQLLESGGGLVQPGGSLRLSCAASGFTFSTYAMNWVRQAPGKGLEWVSRIRSKYNNYATYYADSVKDRFTISRDDSKSTLYLQMNSLRAEDTAVYYCVRHGNFGNSYVSWFAYWGQGTLVTVSSASTKGPSVFPLAPSSKSTSGGTAALGCLVKDYFPEPVTVSWNSGALTSGVHTFPAVLQSSGLYSLSSVVTVPSSSLGTQTYICNVNHKPSNTKVDKKVEPKSCDKTHTCPPCPAPEAAGGPSVFLFPPKPKDTLMISRTPEVTCVVVDVSHEDPEVKFNWYVDGVEVHNAKTKPREEQYNSTYRVVSVLTVLHQDWLNGKEYKCKVSNKALPAPIEKTISKAKGQPREPQVYTLPPCREEMTKNQVSLWCLVKGFYPSDIAVEWESNGQPENNYKTTPPVLDSDGSFFLYSKLTVDKSRWQQGNVFSCSVMHEALHNHYTQKSLSLSPGK

SEQ ID NO: 129 - protein, 477 aa, Artificial Sequence
  Synthetic
EIVMTQSPASLSVSPGERATLSCRASQSVSSNLAWYQQKPGQAPRLLIYGASTRATGIPARVSGGGSGTEFTLTISSLQSEDFAVYYCQQYKNWPFTFGPGTKLEIKGGGGSGGGGSGGGGSGGGGSQVQLVQSGAEVKKPGSSMRVSCKASEDTFSSYAISWVRQAPGQGLEWMGGTAPIFGTTNYAQKFQGRVTITADKSTSTAYMELSSLRSEDTAVYYCARGGPYFDYWGQGTLVTVSSASEPKSSDKTHTCPPCPAPEAAGGPSVFLFPPKPKDTLMISRTPEVTCVVVDVSHEDPEVKFNWYVDGVEVHNAKTKPREEQYNSTYRVVSVLTVLHQDWLNGKEYKCKVSNKALPAPIEKTISKAKGQPREPQVCTLPPSREEMTKNQVSLSCAVKGFYPSDIAVEWESNGQPENNYKTTPPVLDSDGSFFLVSKLTVDKSRWQQGNVFSCSVMHEALHNHYTQKSLSLSPGK

SEQ ID NO: 130 - protein, 455 aa, Artificial Sequence
  Synthetic
EVQLVESGGGLVQPGGSLKLSCAASGFTFSTYAMNWVRQASGKGLEWVGRIRSKYNNYATYYADSVKDRFTISRDDSKNTAYLQMNSLKTEDTAVYYCTRHGNFGNSYVSWFAYWGQGTLVTVSSASTKGPSVFPLAPSSKSTSGGTAALGCLVKDYFPEPVTVSWNSGALTSGVHTFPAVLQSSGLYSLSSVVTVPSSSLGTQTYICNVNHKPSNTKVDKKVEPKSCDKTHTCPPCPAPEAAGGPSVFLFPPKPKDTLMISRTPEVTCVVVDVSHEDPEVKFNWYVDGVEVHNAKTKPREEQYNSTYRVVSVLTVLHQDWLNGKEYKCKVSNKALPAPIEKTISKAKGQPREPQVYTLPPCREEMTKNQVSLWCLVKGFYPSDIAVEWESNGQPENNYKTTPPVLDSDGSFFLYSKLTVDKSRWQQGNVFSCSVMHEALHNHYTQKSLSLSPGK

SEQ ID NO: 131 - protein, 483 aa, Artificial Sequence
  Synthetic
QAVVTQEPSLTVSPGGTVTLTCRSSTGAVTTSNYANWVQQKPGQAPRGLIGGTNKRAPWTPARFSGSLLGDKAALTLLGAQPEDEAEYFCALWYSNLWVFGGGTKLTVLGGGQSGQGGSGGGGSEVQLVESGGGLVQPGGSLKLSCAASGFTFNTYAMNWVRQASGKGLEWVGRIRSKYNNYATYYADSVKDRFTISRDDSKSTLYLQMNSLKTEDTAVYYCVRHGNFGNSYVSWFAYWGQGTLVTVSSASEPKSSDKTHTCPPCPAPEAAGGPSVFLFPPKPKDTLMISRTPEVTCVVVDVSHEDPEVKFNWYVDGVEVHNAKTKPREEQYNSTYRVVSVLTVLHQDWLNGKEYKCKVSNKALPAPIEKTISKAKGQPREPQVYTLPPSREEMTKNQVSLTCLVKGFYPSDIAVEWESNGQPENNYKTTPPVLDSDGSFFLYSKLTVDKSRWQQGNVFSCSVMHEALHNHYTQKSLSLSPGK

SEQ ID NO: 132 - protein, 480 aa, Artificial Sequence
  Synthetic
EIVMTQSPASLSVSPGERATLSCRASQSVSSNLAWYQQKPGQAPRLLIYGASTRATGIPARVSGGGSGTEFTLTISSLQSEDFAVYYCQQYKNWPFTFGPGTKLEIKGGGGSGGGGSGGGGSGGGGSQVQLVQSGAEVKKPGSSMRVSCKASEDTFSSYAISWVRQAPGQGLEWMGGTAPIFGTTNYAQKFQGRVTITADKSTSTAYMELSSLRSEDTAVYYCARGGPYFDYWGQGTLVTVSSGGGASEPKSCDKTHTCPPCPAPELLGGPSVFLFPPKPKDTLMISRTPEVTCVVVDVSHEDPEVKFNWYVDGVEVHNAKTKPREEQYNSTYRVVSVLTVLHQDWLNGKEYKCKVSNKALPAPIEKTISKAKGQPREPQVYTLPPSREEMTKNQVSLTCLVKGFYPSDIAVEWESNGQPENNYKTTPPVLDSDGSFFLYSKLTVDKSRWQQGNVFSCSVMHEALHNHYTQKSLSLSPGK

SEQ ID NO: 133 - protein, 5 aa, Artificial Sequence
  GS_5
GGGGS

SEQ ID NO: 134 - protein, 15 aa, Artificial Sequence
  GS_15
GGGQSGQGGSGGGGS

SEQ ID NO: 135 - protein, 20 aa, Artificial Sequence
  GS_20
GGGGSGGGGSGGGGSGGGGS